European Patent Application EP 4 549 570 A1, published May 7, 2025. Title: LUCIFERASE MUTANT AND USE THEREOF. Applicant: DGI TECH (QING DAO) CO., LIMITED. The sequence listing filed with the application follows.

SEQUENCE LISTING (34 sequences)

SEQ ID NO: 1 - DNA, 540 bp, Artificial
  Gene sequence of wild type Pleuromamma xiphia luciferase (WT Pxluc) containing a signal peptide
atgtatataaaagtttggtttggtctggcttgtctttcattggttctggcccaaccaactgaaaacaagcaggagtctcatattgtagattcagatcttgatggcgaccgtggtaggaagttgcccggaaaaaagcttcctatagaagtactcaaaatcatggaagccaatgccaggagagctggttgcactagaggatgtctcatatgtctttcaaaaatcaagtgtacagccaaaatgaagcgatacattccagggagatgtcatacttatgaaggagataaatctattggacagggaggcataggtggccctattgttgatattcctgaaattattggattcaagaacatggaacccatggatcagttcatcgcacaagttgatctgtgcgccgactgtacaactgggtgcctgaaaggccttgctaatgttaggtgcaatgacttgctgaagaaatggctgcctgacagatgtgctggttttgccgacaaaattcaaaatgaagtggatagtatcaagggcatggctggggatcgc

SEQ ID NO: 2 - protein, 180 aa, Artificial
  amino acid sequence of wild type Pleuromamma xiphia luciferase (WT Pxluc) containing a signal peptide
MYIKVWFGLACLSLVLAQPTENKQESHIVDSDLDGDRGRKLPGKKLPIEVLKIMEANARRAGCTRGCLICLSKIKCTAKMKRYIPGRCHTYEGDKSIGQGGIGGPIVDIPEIIGFKNMEPMDQFIAQVDLCADCTTGCLKGLANVRCNDLLKKWLPDRCAGFADKIQNEVDSIKGMAGDR

SEQ ID NO: 3 - DNA, 489 bp, Artificial
  Gene sequence of the wild type Pleuromamma xiphia luciferase without a signal peptide (WT-NS Pxluc)
caaccaactgaaaacaagcaggagtctcatattgtagattcagatcttgatggcgaccgtggtaggaagttgcccggaaaaaagcttcctatagaagtactcaaaatcatggaagccaatgccaggagagctggttgcactagaggatgtctcatatgtctttcaaaaatcaagtgtacagccaaaatgaagcgatacattccagggagatgtcatacttatgaaggagataaatctattggacagggaggcataggtggccctattgttgatattcctgaaattattggattcaagaacatggaacccatggatcagttcatcgcacaagttgatctgtgcgccgactgtacaactgggtgcctgaaaggccttgctaatgttaggtgcaatgacttgctgaagaaatggctgcctgacagatgtgctggttttgccgacaaaattcaaaatgaagtggatagtatcaagggcatggctggggatcgc

SEQ ID NO: 4 - protein, 163 aa, Artificial
  Amino acid  sequence of the wild type Pleuromamma xiphia luciferase without a signal peptide (WT-NS Pxluc)
QPTENKQESHIVDSDLDGDRGRKLPGKKLPIEVLKIMEANARRAGCTRGCLICLSKIKCTAKMKRYIPGRCHTYEGDKSIGQGGIGGPIVDIPEIIGFKNMEPMDQFIAQVDLCADCTTGCLKGLANVRCNDLLKKWLPDRCAGFADKIQNEVDSIKGMAGDR

SEQ ID NO: 5 - DNA, 627 bp, Artificial
  Gene sequence of Pleuromamma xiphia luciferase containing a signal peptide for pET28a vector (pET28a Pxluc WT)
aagcttgccgccaccatgtatataaaagtttggtttggtctggcttgtctttcattggttctggcccaaccaactgaaaacaagcaggagtctcatattgtagattcagatcttgatggcgaccgtggtaggaagttgcccggaaaaaagcttcctatagaagtactcaaaatcatggaagccaatgccaggagagctggttgcactagaggatgtctcatatgtctttcaaaaatcaagtgtacagccaaaatgaagcgatacattccagggagatgtcatacttatgaaggagataaatctattggacagggaggcataggtggccctattgttgatattcctgaaattattggattcaagaacatggaacccatggatcagttcatcgcacaagttgatctgtgcgccgactgtacaactgggtgcctgaaaggccttgctaatgttaggtgcaatgacttgctgaagaaatggctgcctgacagatgtgctggttttgccgacaaaattcaaaatgaagtggatagtatcaagggcatggctggggatcgcggtggcagtgaaaatctgtattttcagagcggcggccatcatcatcatcatcatggcagctgatgagaattc

SEQ ID NO: 6 - DNA, 586 bp, Artificial
  Gene sequence of Pleuromamma xiphia luciferase containing a signal peptide for pCold vector
caccatgaatcacaaagtgcatatgatgtatataaaagtttggtttggtctggcttgtctttcattggttctggcccaaccaactgaaaacaagcaggagtctcatattgtagattcagatcttgatggcgaccgtggtaggaagttgcccggaaaaaagcttcctatagaagtactcaaaatcatggaagccaatgccaggagagctggttgcactagaggatgtctcatatgtctttcaaaaatcaagtgtacagccaaaatgaagcgatacattccagggagatgtcatacttatgaaggagataaatctattggacagggaggcataggtggccctattgttgatattcctgaaattattggattcaagaacatggaacccatggatcagttcatcgcacaagttgatctgtgcgccgactgtacaactgggtgcctgaaaggccttgctaatgttaggtgcaatgacttgctgaagaaatggctgcctgacagatgtgctggttttgccgacaaaattcaaaatgaagtggatagtatcaagggcatggctggggatcgcggtggcagtgagaacctgtac

SEQ ID NO: 7 - DNA, 531 bp, Artificial
  Gene sequence of Pleuromamma xiphia luciferase without the signal peptide for pCold vector
catgaatcacaaagtgcatatgcaaccaactgaaaacaagcaggagtctcatattgtagattcagatcttgatggcgaccgtggtaggaagttgcccggaaaaaagcttcctatagaagtactcaaaatcatggaagccaatgccaggagagctggttgcactagaggatgtctcatatgtctttcaaaaatcaagtgtacagccaaaatgaagcgatacattccagggagatgtcatacttatgaaggagataaatctattggacagggaggcataggtggccctattgttgatattcctgaaattattggattcaagaacatggaacccatggatcagttcatcgcacaagttgatctgtgcgccgactgtacaactgggtgcctgaaaggccttgctaatgttaggtgcaatgacttgctgaagaaatggctgcctgacagatgtgctggttttgccgacaaaattcaaaatgaagtggatagtatcaagggcatggctggggatcgcggtggcagtgagaacctgta

SEQ ID NO: 8 - DNA, 40 bp, Artificial
  Forward Primer insert-F1（WT Pxluc）
caccatgaatcacaaagtgcatatgtatataaaagtttgg

SEQ ID NO: 9 - DNA, 44 bp, Artificial
  Forward Primer insert-F2 (WT-NS Pxluc)
catgaatcacaaagtgcatatgcaaccaactgaaaacaagcagg

SEQ ID NO: 10 - DNA, 40 bp, Artificial
  Reverse Primer insert-R
gtacaggttctcactgccaccgcgatccccagccatgccc

SEQ ID NO: 11 - DNA, 40 bp, Artificial
  Forward Primer vector-F1
gggcatggctggggatcgcggtggcagtgagaacctgtac

SEQ ID NO: 12 - DNA, 40 bp, Artificial
  Reverse Primer vector-R1 (WT Pxluc)
ccaaacttttatatacatatgcactttgtgattcatggtg

SEQ ID NO: 13 - DNA, 44 bp, Artificial
  Reverse Primer vector-R2 (WT-NS Pxluc)
cctgcttgttttcagttggttgcatatgcactttgtgattcatg

SEQ ID NO: 14 - DNA, 40 bp, Artificial
  Forward Primer F1
  misc_feature (13)..(14): n is a, c, g, or t
gataaatctattnnkcagggaggcataggtggccctattg

SEQ ID NO: 15 - DNA, 40 bp, Artificial
  Reverse Primer R1
  misc_feature (24)..(25): n is a, c, g, or t
tagggccacctatgcctccctgmnnaatagatttatctcc

SEQ ID NO: 16 - DNA, 40 bp, Artificial
  Forward Primer F2
  misc_feature (16)..(17): n is a, c, g, or t
gataaatctattggannkggaggcataggtggccctattg

SEQ ID NO: 17 - DNA, 40 bp, Artificial
  Reverse Primer R2
  misc_feature (21)..(22): n is a, c, g, or t
tagggccacctatgcctccmnntccaatagatttatctcc

SEQ ID NO: 18 - DNA, 40 bp, Artificial
  Forward Primer F3
  misc_feature (19)..(20): n is a, c, g, or t
gataaatctattggacagnnkggcataggtggccctattg

SEQ ID NO: 19 - DNA, 40 bp, Artificial
  Reverse Primer R3
  misc_feature (18)..(19): n is a, c, g,or t
tagggccacctatgccmnnctgtccaatagatttatctcc

SEQ ID NO: 20 - DNA, 40 bp, Artificial
  Forward Primer F4
  misc_feature (22)..(23): n is a, c, g, or t
gataaatctattggacagggannkataggtggccctattg

SEQ ID NO: 21 - DNA, 40 bp, Artificial
  Reverse Primer R4
  misc_feature (15)..(16): n is a, c, g, or t
tagggccacctatmnntccctgtccaatagatttatctcc

SEQ ID NO: 22 - DNA, 40 bp, Artificial
  Forward Primer F5
  misc_feature (13)..(14): n is a, c, g, or t
  misc_feature (16)..(17): n is a, c, g, or t
gataaatctattnnknnkggaggcataggtggccctattg

SEQ ID NO: 23 - DNA, 40 bp, Artificial
  Reverse Primer R5
  misc_feature (21)..(22): n is a, c, g,or t
  misc_feature (24)..(25): n is a, c, g, or t
tagggccacctatgcctccmnnmnnaatagatttatctcc

SEQ ID NO: 24 - DNA, 40 bp, Artificial
  Forward Primer F6
  misc_feature (19)..(20): n is a, c, g, or t
  misc_feature (22)..(23): n is a, c, g, or t
gataaatctattggacagnnknnkataggtggccctattg

SEQ ID NO: 25 - DNA, 40 bp, Artificial
  Reverse Primer R6
  misc_feature (15)..(16): n is a, c, g, or t
  misc_feature (18)..(19): n is a, c, g,or t
tagggccacctatmnnmnnctgtccaatagatttatctcc

SEQ ID NO: 26 - DNA, 52 bp, Artificial
  Forward Primer F7
  misc_feature (19)..(20): n is a, c, g, or  t
  misc_feature (22)..(23): n is a, c, g, or t
  misc_feature (25)..(26): n is a, c, g,or t
  misc_feature (28)..(29): n is a, c, g, or t
gaaggagataaatctattnnknnknnknnkataggtggccctattgttgata

SEQ ID NO: 27 - DNA, 52 bp, Artificial
  Reverse Primer R7
  misc_feature (18)..(19): n is a, c, g, or t
  misc_feature (21)..(22): n is a, c, g,or t
  misc_feature (24)..(25): n is a, c, g, or t
  misc_feature (27)..(28): n is a, c, g, or t
caatagggccacctatmnnmnnmnnmnnaatagatttatctccttcataagt

SEQ ID NO: 28 - DNA, 585 bp, Artificial
  Gene sequence of Pleuromamma xiphia luciferase containing a signal peptide for pEE12.4 vector
atgtatataaaagtttggtttggtctggcttgtctttcattggttctggcccaccaccaccaccatcacggcagccaaccaactgaaaacaagcaggagtctcatattgtagattcagatcttgatggcgaccgtggtaggaagttgcccggaaaaaagcttcctatagaagtactcaaaatcatggaagccaatgccaggagagctggttgcactagaggatgtctcatatgtctttcaaaaatcaagtgtacagccaaaatgaagcgatacattccagggagatgtcatacttatgaaggagataaatctattggacagggaggcataggtggccctattgttgatattcctgaaattattggattcaagaacatggaacccatggatcagttcatcgcacaagttgatctgtgcgccgactgtacaactgggtgcctgaaaggccttgctaatgttaggtgcaatgacttgctgaagaaatggctgcctgacagatgtgctggttttgccgacaaaattcaaaatgaagtggatagtatcaagggcatggctggggatcgcggctccggactgaatgatatc

SEQ ID NO: 29 - DNA, 36 bp, Artificial
  Forward Primer insert-F
caccaccatcacggcagccaaccaactgaaaacaag

SEQ ID NO: 30 - DNA, 37 bp, Artificial
  Reverse Primer insert-R
gatatcattcagtccggagccgcgatccccagccatg

SEQ ID NO: 31 - DNA, 37 bp, Artificial
  Forward primer
catggctggggatcgcggctccggactgaatgatatc

SEQ ID NO: 32 - DNA, 36 bp, Artificial
  Reverse primer
cttgttttcagttggttggctgccgtgatggtggtg

SEQ ID NO: 33 - DNA, 40 bp, Artificial
  Forward primer
gataaatctattggacaggcgcctataggtggccctattg

SEQ ID NO: 34 - DNA, 40 bp, Artificial
  Reverse primer
tagggccacctataggcgcctgtccaatagatttatctcc